European Patent Application EP 4 269 591 A1, published November 1, 2023. Title: The assay system for assessing immunotoxicity caused by suppression of cell proliferation. Applicant: TOHOKU UNIVERSITY. The sequence listing filed with the application follows.

SEQUENCE LISTING (3 sequences)

SEQ ID NO: 1 - DNA, 1501 bp, Homo sapiens
ggtcagggactggagtcctgtgggtgctttttaagcaaagattatcaccaggcaggctaaacttagcaaccggcttttagctagaagggcagggggctggtgtcaggttatgctgggccagcaaagaggcccgggatccccctcccatgcacctgctgatgggccaaggccaccccaccccacccccttccttacaagtgttcagcaccctcccatcccacactcacaaacctggccctctgccctcctaccagaagaatggatcccctgtgggagggggcaggggacctgttcccaccgtgtgcccaagacctcttttcccactttttccctcttcttgactcaccctgccctcaatatcccccggcgcagccagtgaaagggagtccctggctcctggctcgcctgcacgtcccagggcggggagggacttccgccctcacgtcccgctcttcgccccaggctggatggaatgaaaggcacactgtctctctccctaggcagcacagcccacaggtttccaggagtgcctttgtgggaggcctctgggcccccaccagccatcctgtcctccgcctggggccccagcccggagagagccgctggtgcacacagggccgggattgtctgccctaattatcaggtccaggctacagggctgcaggacatcgtgaccttccgtgcagaaacctccccctccccctcaagccgcctcccgagcctccttcctctccaggcccccagtgcccagtgcccagtgcccagcccaggcctcggtcccagagatgccaggagccaggagatggggagggggaagtgggggctgggaaggaaccacgggcccccgcccgaggcccatgggcccctcctaggcctttgcctgagcagtccggtgtcactaccgcagagcctcgaggagaagttccccaactttcccgcctctcagcctttgaaagaaagaaaggggagggggcaggccgcgtgcagccgcgagcggtgctgggctccggctccaattccccatctcagtcgttcccaaagtcctcctgtttcatccaagcgtgtaagggtccccgtccttgactccctagtgtcctgctgcccacagtccagtcctgggaaccagcaccgatcacctcccatcgggccaatctcagtcccttcccccctacgtcggggcccacacgctcggtgcgtgcccagttgaaccaggcggctgcggaaaaaaaaaagcggggagaaagtagggcccggctactagcggttttacgggcgcacgtagctcaggcctcaagaccttgggctgggactggctgagcctggcgggaggcggggtccgagtcaccgcctgccgccgcgcccccggtttctataaattgagcccgcagcctcccgcttcgctctctgctcctcctgttcgacagtcagccgcatcttcttttgcgtcgccaggtgaagacgggcggagagaaacccgggaggctagggacggcctgaaggc

SEQ ID NO: 2 - DNA, 3282 bp, Homo sapiens
agatggatgatgccttccttgaatcatcagctaccaccgacagagtgaagtgagatggaatagtgggcacaatctcattcatcctactctatgtagcctaatgggtccagaatttattatcactattttacactggaaaaaagatgagattatgaggggtcagggaggctttgagtttttgctctaacttcaccactaattaagaatgtgatcttgggtaagccactttaacctctgtaaatgtcaaatttcttatcagtaaaatgtgactatacaagacaataaatttgaaaatactttgcaaaattgaaagtaccatggaaataattcttcaatcccaaaaggttatgaacattattaaaatttgccacatggaagagcacacaccacagagacataactgtgatcataaacagatttacaaaagtggtgtttcattatggagggccatagggctgataaagacaaatgcatcaccaagctatgtccgagctcattcagatttttacaggaaacacagagcttctagctgaattatctctggatggtgtggaaattgtccaacacgttcctaatttcaaagaaacagaactgaatcttgaaaacccaagaggcctttacagaaactgacaagagatgaattaatataggtatcaagctacagaccaaattaaagttttacaaaactttgaaagagggtcagaaagaagaaacttatgggaagcagagtcctggaaagtcagctttgatggagtgacaatatgtgcaacacagtgagcaatctcttaggtaggcagcttcagggatgggggttgccctttgaaaggacttgggccactcttgagtctaagaggctaagtcacaaacaatgctaagcaactaaaaatagcttcttgtttaatagtaaaattctgcatagtaaaaggagaagcagggggtatgacacacgtggtagttagcagtctactagtgactttactgccacaaccagaaaagccagctgatgtgtcagacgtgagaaagcgaaagtatgtcacagcgaatgtagcttttccacacgtatttcaagaaagaaatgaaaaagccaacttctataatggtgcctactgtgcattaacagagataaactaggggtctaagaactcagttttctacagggtcccagaagtatagccatatattgccccattctctaatggaaatagccagagaaatagaaatatcaagactggagaacatcaaatacctcattggaaaagcccccacataggaaaatgtgtgggcttgaattcttccattctggaagggtaaaggcctgagtgatgatgctgggattagacactgaaactctttagagaagcaaaacaagtataataaagctgtactttattatattaaataaataacacacagactaccaaatagcctgccccttataacagcgttaatgtgattttgatctgaaatgtatagagacattttgcattttttcgtataaaaagttcatgagatttggccctaatctgaccttttcttcatttttttttctacttgagggactataatctttatttttaaatttgttttatattctccgaacattacctaacgcatagaaaactcttattgaaccatttttctctgttctttgtaaaatattacatttgactgttccttagactgctttaatcattcctgcctatgcaccctcctcaaaatccagtttaaattaattgttccttattcaagattccttatatccacctcccttggggcagcaatcacctatcacccaggactacacttgtgtatgtacatatcttccctattacaaatcaggttctttgaaaaaatacaaatggtaagagagtggatttttggagtcagaacattctcttttcaaatccttcttctgccccttactggcaataagggctgagtgacctagagcaaattacttaacttctctgagcctcagttttctaatctgcaaaataggagccatcacttcacaagtctgtaagacttatattagactaagtgcctgcctgtacactgttctcttttctctctttctatatacctgaaggcattataggtgctagatgtctgtttaaagaccagacaatattgtcttaaaaaaacaaacaaaaacacagacaataccatctttaaaaaaaaaaaaaaagtccaggtaagaaataaataaggccatagaatggaagctttacaaggactctctctgagacaggatctcctcaagtgtccccaggttaaattagaagtatatatccgtacaattgttcagccagtttgtgcactgtactgaggatgaatgaacacctatcctaaatatcctagtcttctgactaaaaacaagatcatatttcataacgattattgttacattcatagtgtcccaggtgatttagaggataaataaaaatccattaaagaggtaaagacataaaaacgagaaacatggactggtttacacataacacatacaaagtctattataaaactagcatcagtatccttgaatgcaaacctttttctgagtatttaacaatcgcaccctttaaaaaatgtacaatagacattaagagacttaaacagatatataatcattttaaattaaaatagcgttaaacagtacctcaagctcaataagcattttaagtattctaatcttagtatttctctagctgacatgtaagaagcaatctatcttattgtatgcaattagctcattgtgtggataaaaaggtaaaaccattctgaaacaggaaaccaatacacttcctgttttatcaacaaatctaaacatttattcttttcatctgtttactcttgctcttgtccaccacaatatgctattcacatgttcagtgtagttttatgacaaagaaaattttctgagttacttttgtatccccacccccttaaagaaaggaggaaaaactgtttcatacagaaggcgttaattgcatgaattagagctatcacctaagtgtgggctaatgtaacaaagagggatttcacctacatccattcagtcagtctttgggggtttaaagaaattccaaagagtcatcagaagaggaaaaatgaaggtaatgttttttcagacaggtaaagtctttgaaaatatgtgtaatatgtaaaacattttgacacccccataatatttttccagaattaacagtataaattgcatctcttgttcaagagttccctatcactctctttaatcactactcacagtaacctcaactcctg

SEQ ID NO: 3 - DNA, 5076 bp, Homo sapiens
acacaatacatatgtcaatgtgtgtatttccctctgaccaataataagtcctcttaacgatatgaaccacctggagaggatgtacatggagaaaaggtggggaatatggatacctattctacctattcagcaacaagaacaggaatcaatcctagcttccaatgtggtgacatatgctcctaccggattgtctcactgctaacttctttgtaacccctaaagctatggatatctagtaggcattcaattcaataagcacatattaattaattgaaattgggatataaaccaacattttcacaatagaacttttcatccttctttggaaaccccatatcaatcgaagtatttggcacttggtgcattaaaattccttgtggaacaaaaatacaaccttcaaagcaggaccatgaatctctggattatcaatacacaatcccatctgatataaaattaagaatattgtaatctgatgattgtactgtgtaagtagcataccttctatattctttgaaccactcctcaaaaatggccagaaggcacaaaagaaaaggggggattcagaaaaatcttcctctaacttacgggattttatgagtcaaattgcggggaaaatctgactccgtgtggacttctattctgtatgtcatgcttcttccgtaggtttggcttgcatgatgtcaggagttccggaagtcaaaatagcgtgggggcatggatccaatattgactcatattgagtggaagaaatctacgccaaagtctggatgagataatttggttgtgagtgctaggatgtgactgctgatgacagaggaaaagggaaaccaaggtgtaagttttggcttactgactacctactcagttaagactgaggatagcatgagatatgattgaaatgttgctgatgtgtcatgtataaccatagccagttttcagaaaaaaagtctagttgaaaagaaaaaagaaagttttcagcccctctgttttagtaatatggtcacaccttggctcctgatggctttgcaaaacttttaaagtatatcttgatggtgacttattctgcagtctcagaactggccaaaccaacaaagtgtgaaacctctagtttgcatgtgcaacaaaaggtgttttacaggcagaaaagagagagaaatttctttgtttgcaaagttgacaagacaggaaaagatcacaaacgtatatacttattgtagtgataatgttctgaacaaaagaatcatatgttgaaagatgaaaatctaatagcagatgtttcactgccagtctggaatgcaggaccagctgcataatttgtggaaacaagtgcaaaacgaaaatgtgtgtcctttgtttgaagagttattagaaatttcaaggaagtgacaacagagcattaaaccaagtgtgggctgttctaagttcagggtcctgtcagactgcacaggttgcatgtccatgaagtcaggttggctgggatgtctaggcaaaaatttcaaaaatatatttcagaaacaatttcaaattatacttgcagtcttactatgttttaaggaattaaagtgtgattactatctcacaaattctacagaagaaaaaatctcagaaactaaagcctgatagggtgtagttatttgaattcacatatctaacgtagaggtacatgcaatcatctcaatggatattgatagattgggggatggattgactaagggttccatcctctttgggaagatcttggatttagactcagttctgcattagccagttgaatgaatttaagcacatcacttgtctttctgggtctggatttacaaatctaaaaggtaaggggttgaccatagataatctataattccataattctgtgcttggccatgccatcaagagttattagagcttggattttagccgtgtaattactctttgtaaacagttgccacactgtaaacatattcttaatataatctgttattttgaataggcattctcaatttacaagtggctaggcagtatatcattccctcttatggatcccactattcttaactcctcaatcctagtactacattccagtggagcaatcaaggaccaggcagaactaatttttacttatttccagacagttgggaacattccttccagtgactcagaggttgggcattggaaggtattgagaacctgcaaagtgtctcaggctctgacccaaatccctgtgccacctgcaagcacgttctctggacgtaatttttcttgagcagagcaacagtagagctttgtatgcaacaatgtaatttttacattcttcacttgcttaacatgaggtttggttccacataaatgttttgatcttatttattctttgggaagatcgcccctcaaagagctttctggcttttttttcccacataaaagaatacacgaaattgtcgcagtcagcaagtgttggctaaagagacacagcatcatgtttctaacattaatcataaatattatttaattaaaaactagtttcttacaggttaggcctgataacatcggaattagaatttgagggcaaataactcaaaagagagccttaggcaagcattcgaatttacatttattcagtgctctttatgagcaaatctccatgctaaaatattttagggaagagaaagccatcataaaagcaatgaaacaatttctgattttcagaaactcaatctaacatggcagaagacacgcgaatagctatcttcaatcaagattgaggaatcagaactcttagaaaagtataaaccaagacttgtatagagaatctaagattaattttaaggaggataattttggaaaaactcagggagatggtaatttttaagccgggcttggatggatggctactactctcaggggcacaaatgaggggaaaaagaactcaagaccaaagaaacagcatgagcaaaggtccagggtacttttttttttaaagaaatgactaggccgggtgcggtggctcacgcctgtaatcccagcactttgggaggccaaggcgggcggatcacgaggtcaggagatcgagaccatcctgattaacacagtgaaaccccgtctgtactaaaaatagcacaaaaaaaaaaaaaaaaaattagccgggcgtggcgagtgcctgtagtcccagctactcgggaggctgaggcgggagaatggcgtgaatccgggaggcagagcttgcagtgagccgagattgcgccactgcactccagcctgggtgacagagcaagactccgtctcaaaaaaaaaaaaaaaagaaatgactagtcatccaatgtgccaaaataataataaacttttattagtgattactatatgccaggaaaaattcctagcactttatgaggattacctgatttaattttcaactgaagcatggaagaagatactattatcaagccagttttacaggtaaggagactgagtcatagaagatttaagaagctaactcacaatcatatagctagatagtagaggagtcaggaatcaagtttgccccataactgcaatactgttatgtacacagtacaggtagaaatgcaaagtgggtttgaaccaaagagtggagggctttttgtgccatcccaaagtgttgtacttcataaataaattacaaaggaggagaaagaatcctatttttttttgtatctgaaagacaaagaaataaaaagttaaaaagattctctgttagtactgattatttggaacaataaattgtttagagctatgctgttcaatatagtagcacctagcagtatgtgcccattaagcgtttgaaatacgactagaccaaattgagatgcaccgtaggcttaaaatatacactgtatttctttccttttttctttttttctttttttttttttgagacggaatcttactctgtcacctaggctggagtgtagtggcgcgatctcggctcactgcaacctccaccttctgggttcaagccattctcctgcctcagcctccctagtagctgagattacaggcatacaccaccatgcctggctaatttttttgtatttttagtagagatggggtttcaccatattggctaggctggtctcaaactcctgaccttgtgatccacccgcctcaacctcccaaagtgctgggattacaggtgtgagccactgcgtctggaactccccctgggaatattctctacactgtatttcaaggatttaatatgacaaaaagaatgtcaaataccttattaacaatgtagtatattgatgcatactgaagtactatttgggatatattggtttaaatacaatatattttaaaattatatttaccttttaaaaaaacttttattaatgaggctactagatcatttaaatttacctgtgtggcttgtattgtatttctactgggcagtgctgatctagagcaatttgaaacttgtggtagatattttactaaccaactctgatgaaggacttcctcaccaaattgttcttttaaccgcattctttccttgctttctggtcatttgcaagaaaaattttaaaaggctgcccctttgtaaaggtttgagaggccctagaatttcgtttttcacttgttcccaaccacaagcaaatgatcaatgtgctttgtgaatgaagagtcaacattttaccagggcgaagtggggaggtacaaaaaaatttccagtccttgaatggtgtgaagtaaaagtgccttcaaagaatcccaccagaatggcacaggtgggcataatgggtctgtctcatcgtcaaaggacccaaggagtctaaaggaaactctaactacaacacccaaatgccacaaaaccttagttattaatacaaactatcatccctgcctatctgtcaccatctcatcttaaaaaacttgtgaaaatacgtaatcctcaggagacttcaattaggtataaataccagcagccagaggaggtgcagcacattgttctgatcatctgaagatcagctattagaagagaaagatcagttaagtcctttggacctgatcagcttgatacaagaactactgatttcaacttctttggct